European Patent Application EP 4 674 970 A2, published January 7, 2026. Title: COMPOSITIONS AND METHODS FOR ENHANCING HOMOLOGOUS RECOMBINATION. Applicant: Life Technologies Corporation. Application EP. The sequence listing filed with the application follows.

SEQUENCE LISTING (127 sequences)

SEQ ID NO: 1 - RNA, 104 nt, synthetic construct
  source 1..104: mol_type = other RNA; note = Description of Artificial Sequence: Synthetic polynucleotide
gcatttcggtatgcatatgaatgagttttagagctagaaatagcaagttaaaataaggctagtccgttatcaacttgaaaaagtggcaccgagtcggtgctttt

SEQ ID NO: 2 - DNA, 23 bp, synthetic construct
  source 1..23: mol_type = other DNA; note = Description of Artificial Sequence: Synthetic oligonucleotide
cgtaaagccatacgtatactacc

SEQ ID NO: 3 - DNA, 23 bp, synthetic construct
  modified_base 21: mod_base = OTHER; note = a, c, t, g, unknown or other
  source 1..23: mol_type = other DNA; note = Description of Artificial Sequence: Synthetic oligonucleotide
gcatttcggtatgcatatgangg

SEQ ID NO: 4 - DNA, 48 bp, synthetic construct
  source 1..48: mol_type = other DNA; note = Description of Artificial Sequence: Synthetic oligonucleotide
tcgtgaccaccctgacccacggcgtgcagtgcttcagccgctaccccg

SEQ ID NO: 5 - DNA, 48 bp, synthetic construct
  source 1..48: mol_type = other DNA; note = Description of Artificial Sequence: Synthetic oligonucleotide
tcgtgaccaccctgacctacggcgtgcagtgcttcagccgctaccccg

SEQ ID NO: 6 - DNA, 66 bp, synthetic construct
  source 1..66: mol_type = other DNA; note = Description of Artificial Sequence: Synthetic oligonucleotide
tcgtgaccaccctgacctacggcgtgcagtgcttcagcggcgtgcagtgcttcagccgctaccccg

SEQ ID NO: 7 - DNA, 38 bp, synthetic construct
  source 1..38: mol_type = other DNA; note = Description of Artificial Sequence: Synthetic oligonucleotide
tcgtgactacggcgtgcagtgcttcagccgctaccccg

SEQ ID NO: 8 - DNA, 47 bp, synthetic construct
  source 1..47: mol_type = other DNA; note = Description of Artificial Sequence: Synthetic oligonucleotide
tcgtgaccaccctgaccacggcgtgcagtgcttcagccgctaccccg

SEQ ID NO: 9 - DNA, 38 bp, synthetic construct
  source 1..38: mol_type = other DNA; note = Description of Artificial Sequence: Synthetic oligonucleotide
tcgaggccacggcgtgcagtgcttcagccgctaccccg

SEQ ID NO: 10 - DNA, 33 bp, synthetic construct
  source 1..33: mol_type = other DNA; note = Description of Artificial Sequence: Synthetic oligonucleotide
tctacggcgtgcagtgcttcagccgctaccccg

SEQ ID NO: 11 - DNA, 32 bp, synthetic construct
  source 1..32: mol_type = other DNA; note = Description of Artificial Sequence: Synthetic oligonucleotide
tcgtggcgtgcagtgcttcagccgctaccccg

SEQ ID NO: 12 - DNA, 31 bp, synthetic construct
  source 1..31: mol_type = other DNA; note = Description of Artificial Sequence: Synthetic oligonucleotide
tcgtgcgtgcagtgcttcagccgctaccccg

SEQ ID NO: 13 - DNA, 22 bp, synthetic construct
  source 1..22: mol_type = other DNA; note = Description of Artificial Sequence: Synthetic oligonucleotide
tcgtgaccaagccgctaccccg

SEQ ID NO: 14 - DNA, 14 bp, synthetic construct
  source 1..14: mol_type = other DNA; note = Description of Artificial Sequence: Synthetic oligonucleotide
tcgtgaccaccccg

SEQ ID NO: 15 - DNA, 20 bp, synthetic construct
  source 1..20: mol_type = other DNA; note = Description of Artificial Sequence: Synthetic oligonucleotide
gaccaccctgacccacggcg

SEQ ID NO: 16 - DNA, 50 bp, synthetic construct
  source 1..50: mol_type = other DNA; note = Description of Artificial Sequence: Synthetic oligonucleotide
gaccaccctgaccgactacaaagacgatgacgacaagaattcttacggcg

SEQ ID NO: 17 - DNA, 50 bp, synthetic construct
  source 1..50: mol_type = other DNA; note = Description of Artificial Sequence: Synthetic oligonucleotide
gaccaccctgcccgactacaaagacgatgacgacaagaattcttacggcg

SEQ ID NO: 18 - DNA, 49 bp, synthetic construct
  source 1..49: mol_type = other DNA; note = Description of Artificial Sequence: Synthetic oligonucleotide
gaccaccctgccgactacaaagacgatgacgacaagaattcttacggcg

SEQ ID NO: 19 - DNA, 73 bp, synthetic construct
  source 1..73: mol_type = other DNA; note = Description of Artificial Sequence: Synthetic oligonucleotide
gaccaccctggcctgcaccctcgtgacaccctgaccgactacaaagacgatgacgacaagtattcttacggcg

SEQ ID NO: 20 - DNA, 44 bp, synthetic construct
  source 1..44: mol_type = other DNA; note = Description of Artificial Sequence: Synthetic oligonucleotide
gaccaccctgaccgactacaaagacgacaagaattcttacggcg

SEQ ID NO: 21 - DNA, 35 bp, synthetic construct
  source 1..35: mol_type = other DNA; note = Description of Artificial Sequence: Synthetic oligonucleotide
gaccgactacaaagacgacaagaattcttacggcg

SEQ ID NO: 22 - DNA, 31 bp, synthetic construct
  source 1..31: mol_type = other DNA; note = Description of Artificial Sequence: Synthetic oligonucleotide
gaccgacgatgacgacaaaattcttacggcg

SEQ ID NO: 23 - DNA, 10 bp, synthetic construct
  source 1..10: mol_type = other DNA; note = Description of Artificial Sequence: Synthetic oligonucleotide
gaccacggcg

SEQ ID NO: 24 - DNA, 12 bp, synthetic construct
  source 1..12: mol_type = other DNA; note = Description of Artificial Sequence: Synthetic oligonucleotide
gaccccacggcg

SEQ ID NO: 25 - skipped

SEQ ID NO: 26 - protein, 7 aa, synthetic construct
  source 1..7: note = Description of Artificial Sequence: Synthetic peptide
VTTFTYG

SEQ ID NO: 27 - DNA, 21 bp, synthetic construct
  source 1..21: mol_type = other DNA; note = Description of Artificial Sequence: Synthetic oligonucleotide
  CDS 1..21: protein_id = 26; translation = VTTFTYG
gtgaccaccttcacctacggc

SEQ ID NO: 28 - protein, 5 aa, synthetic construct
  source 1..5: note = Description of Artificial Sequence: Synthetic peptide
VTTYG

SEQ ID NO: 29 - DNA, 15 bp, synthetic construct
  source 1..15: mol_type = other DNA; note = Description of Artificial Sequence: Synthetic oligonucleotide
  CDS 1..15: protein_id = 28; translation = VTTYG
gtgaccacctacggc

SEQ ID NO: 30 - protein, 4 aa, synthetic construct
  source 1..4: note = Description of Artificial Sequence: Synthetic peptide
LTHG

SEQ ID NO: 31 - DNA, 12 bp, synthetic construct
  source 1..12: mol_type = other DNA; note = Description of Artificial Sequence: Synthetic oligonucleotide
  CDS 1..12: protein_id = 30; translation = LTHG
ctgacccacggc

SEQ ID NO: 32 - protein, 4 aa, synthetic construct
  source 1..4: note = Description of Artificial Sequence: Synthetic peptide
LTYG

SEQ ID NO: 33 - DNA, 12 bp, synthetic construct
  source 1..12: mol_type = other DNA; note = Description of Artificial Sequence: Synthetic oligonucleotide
  CDS 1..12: protein_id = 32; translation = LTYG
ctgacctacggc

SEQ ID NO: 34 - protein, 887 aa, Natronobacterium gregoryi
MTVIDLDSTTTADELTSGHTYDISVTLTGVYDNTDEQHPRMSLAFEQDNGERRYITLWKNTTPKDVFTYDYATGSTYIFTNIDYEVKDGYENLTATYQTTVENATAQEVGTTDEDETFAGGEPLDHHLDDALNETPDDAETESDSGHVMTSFASRDQLPEWTLHTYTLTATDGAKTDTEYARRTLAYTVRQELYTDHDAAPVATDGLMLLTPEPLGETPLDLDCGVRVEADETRTLDYTTAKDRLLARELVEEGLKRSLWDDYLVRGIDEVLSKEPVLTCDEFDLHERYDLSVEVGHSGRAYLHINFRHRFVPKLTLADIDDDNIYPGLRVKTTYRPRRGHIVWGLRDECATDSLNTLGNQSVVAYHRNNQTPINTDLLDAIEAADRRVVETRRQGHGDDAVSFPQELLAVEPNTHQIKQFASDGFHQQARSKTRLSASRCSEKAQAFAERLDPVRLNGSTVEFSSEFFTGNNEQQLRLLYENGESVLTFRDGARGAHPDETFSKGIVNPPESFEVAVVLPEQQADTCKAQWDTMADLLNQAGAPPTRSETVQYDAFSSPESISLNVAGAIDPSEVDAAFVVLPPDQEGFADLASPTETYDELKKALANMGIYSQMAYFDRFRDAKIFYTRNVALGLLAAAGGVAFTTEHAMPGDADMFIGIDVSRSYPEDGASGQINIAATATAVYKDGTILGHSSTRPQLGEKLQSTDVRDIMKNAILGYQQVTGESPTHIVIHRDGFMNEDLDPATEFLNEQGVEYDIVEIRKQPQTRLLAVSDVQYDTPVKSIAAINQNEPRATVATFGAPEYLATRDGGGLPRPIQIERVAGETDIETLTRQVYLLSQSHIQVHNSTARLPITTAYADQASTHATKGYLVQTGAFESNVGFL

SEQ ID NO: 35 - DNA, 97 bp, synthetic construct
  source 1..97: mol_type = other DNA; note = Description of Artificial Sequence: Synthetic oligonucleotide
catctgcaccaccggcaagctgcccgtgccctggcccaccctcgtgaccaccttcacctacggcgtgcagtgcttcgcccgctaccccgaccacatg

SEQ ID NO: 36 - DNA, 97 bp, synthetic construct
  source 1..97: mol_type = other DNA; note = Description of Artificial Sequence: Synthetic oligonucleotide
catgtggtcggggtagcgggcgaagcactgcacgccgtaggtgaaggtggtcacgagggtgggccagggcacgggcagcttgccggtggtgcagatg

SEQ ID NO: 37 - DNA, 97 bp, synthetic construct; identical to SEQ ID NO: 36
  source 1..97: mol_type = other DNA; note = Description of Artificial Sequence: Synthetic oligonucleotide

SEQ ID NO: 38 - DNA, 79 bp, synthetic construct
  source 1..79: mol_type = other DNA; note = Description of Artificial Sequence: Synthetic oligonucleotide
catgtggtcggggtagcgggcgaagcactgcacgccgtaggtgaaggtggtcacgagggtgggccagggcacgggcagc

SEQ ID NO: 39 - DNA, 79 bp, synthetic construct; identical to SEQ ID NO: 38
  source 1..79: mol_type = other DNA; note = Description of Artificial Sequence: Synthetic oligonucleotide

SEQ ID NO: 40 - DNA, 60 bp, synthetic construct
  source 1..60: mol_type = other DNA; note = Description of Artificial Sequence: Synthetic oligonucleotide
cggggtagcgggcgaagcactgcacgccgtaggtgaaggtggtcacgagggtgggccagg

SEQ ID NO: 41 - DNA, 60 bp, synthetic construct; identical to SEQ ID NO: 40
  source 1..60: mol_type = other DNA; note = Description of Artificial Sequence: Synthetic oligonucleotide

SEQ ID NO: 42 - DNA, 40 bp, synthetic construct
  source 1..40: mol_type = other DNA; note = Description of Artificial Sequence: Synthetic oligonucleotide
ggcgaagcactgcacgccgtaggtgaaggtggtcacgagg

SEQ ID NO: 43 - DNA, 40 bp, synthetic construct; identical to SEQ ID NO: 42
  source 1..40: mol_type = other DNA; note = Description of Artificial Sequence: Synthetic oligonucleotide

SEQ ID NO: 44 - DNA, 100 bp, synthetic construct
  source 1..100: mol_type = other DNA; note = Description of Artificial Sequence: Synthetic polynucleotide
accggcaagctgcccgtgccctggcccaccctcgtgaccaccctgacctacggcgtgcagtgcttcagccgctaccccgaccacatgaagcagcacgact

SEQ ID NO: 45 - DNA, 99 bp, synthetic construct
  source 1..99: mol_type = other DNA; note = Description of Artificial Sequence: Synthetic oligonucleotide
accggcaagctgcccgtgccctggcccaccctctgaccaccctgacctacggcgtgcagtgcttcagccgctaccccgaccacatgaagcagcacgact

SEQ ID NO: 46 - DNA, 90 bp, synthetic construct
  source 1..90: mol_type = other DNA; note = Description of Artificial Sequence: Synthetic oligonucleotide
gcaagctgcccgtgccctggcccaccctcgtgaccaccctgacctacggcgtgcagtgcttcagccgctaccccgaccacatgaagcagc

SEQ ID NO: 47 - DNA, 90 bp, synthetic construct; identical to SEQ ID NO: 46
  source 1..90: mol_type = other DNA; note = Description of Artificial Sequence: Synthetic oligonucleotide

SEQ ID NO: 48 - DNA, 80 bp, synthetic construct
  source 1..80: mol_type = other DNA; note = Description of Artificial Sequence: Synthetic oligonucleotide
gctgcccgtgccctggcccaccctcgtgaccaccctgacctacggcgtgcagtgcttcagccgctaccccgaccacatga

SEQ ID NO: 49 - DNA, 80 bp, synthetic construct; identical to SEQ ID NO: 48
  source 1..80: mol_type = other DNA; note = Description of Artificial Sequence: Synthetic oligonucleotide

SEQ ID NO: 50 - DNA, 70 bp, synthetic construct
  source 1..70: mol_type = other DNA; note = Description of Artificial Sequence: Synthetic oligonucleotide
cccgtgccctggcccaccctcgtgaccaccctgacctacggcgtgcagtgcttcagccgctaccccgacc

SEQ ID NO: 51 - DNA, 70 bp, synthetic construct; identical to SEQ ID NO: 50
  source 1..70: mol_type = other DNA; note = Description of Artificial Sequence: Synthetic oligonucleotide

SEQ ID NO: 52 - DNA, 60 bp, synthetic construct
  source 1..60: mol_type = other DNA; note = Description of Artificial Sequence: Synthetic oligonucleotide
gccctggcccaccctcgtgaccaccctgacctacggcgtgcagtgcttcagccgctaccc

SEQ ID NO: 53 - DNA, 60 bp, synthetic construct; identical to SEQ ID NO: 52
  source 1..60: mol_type = other DNA; note = Description of Artificial Sequence: Synthetic oligonucleotide

SEQ ID NO: 54 - DNA, 50 bp, synthetic construct
  source 1..50: mol_type = other DNA; note = Description of Artificial Sequence: Synthetic oligonucleotide
cccaccctcgtgaccaccctgacctacggcgtgcagtgcttcagccgcta

SEQ ID NO: 55 - DNA, 50 bp, synthetic construct; identical to SEQ ID NO: 54
  source 1..50: mol_type = other DNA; note = Description of Artificial Sequence: Synthetic oligonucleotide

SEQ ID NO: 56 - DNA, 80 bp, synthetic construct
  source 1..80: mol_type = other DNA; note = Description of Artificial Sequence: Synthetic oligonucleotide
gcgtatcaatggatacttacattgactaatccaaactagtgctcattgaccggaaactgttctggaccaatctctttctc

SEQ ID NO: 57 - DNA, 83 bp, synthetic construct
  source 1..83: mol_type = other DNA; note = Description of Artificial Sequence: Synthetic oligonucleotide
gcaatccagtgaatccttgaggtgtaacgtggagccagtaaggcggctacatatctttagtggtgcccatggaccagaaaaag

SEQ ID NO: 58 - DNA, 81 bp, synthetic construct
  source 1..81: mol_type = other DNA; note = Description of Artificial Sequence: Synthetic oligonucleotide
ctgcacggggctgctggcgctcacatttcctattcctggattgatactagagccgctgcctcctcgtagaagctccgacag

SEQ ID NO: 59 - DNA, 98 bp, synthetic construct
  source 1..98: mol_type = other DNA; note = Description of Artificial Sequence: Synthetic oligonucleotide
ctgaccttgccttcatgtgattcagccccagtccattaccctgtgtaggactgagaaatgcaagactctggctagagttccttcttccatctcccttc

SEQ ID NO: 60 - DNA, 98 bp, synthetic construct
  source 1..98: mol_type = other DNA; note = Description of Artificial Sequence: Synthetic oligonucleotide
ctgaccttgccttcatgtgattcagccccagtccattacactgtgtaggactgagaaatgcaagactctggctagagttccttcttccatctcccttc

SEQ ID NO: 61 - DNA, 97 bp, synthetic construct
  source 1..97: mol_type = other DNA; note = Description of Artificial Sequence: Synthetic oligonucleotide
ctgaagttcatctgcaccaccggcaagctgcccgtgccctggcccaccctcgtgaccaccttcacctacggcgtgcagtgcttcgcccgctaccccg

SEQ ID NO: 62 - DNA, 97 bp, synthetic construct
  source 1..97: mol_type = other DNA; note = Description of Artificial Sequence: Synthetic oligonucleotide
cggggtagcgggcgaagcactgcacgccgtaggtgaaggtggtcacgagggtgggccagggcacgggcagcttgccggtggtgcagatgaacttcag

SEQ ID NO: 63 - DNA, 97 bp, synthetic construct
  source 1..97: mol_type = other DNA; note = Description of Artificial Sequence: Synthetic oligonucleotide
ccgtgccctggcccaccctcgtgaccaccttcacctacggcgtgcagtgcttcgcccgctaccccgaccacatgaagcagcacgacttcttcaagtc

SEQ ID NO: 64 - DNA, 97 bp, synthetic construct
  source 1..97: mol_type = other DNA; note = Description of Artificial Sequence: Synthetic oligonucleotide
gacttgaagaagtcgtgctgcttcatgtggtcggggtagcgggcgaagcactgcacgccgtaggtgaaggtggtcacgagggtgggccagggcacgg

SEQ ID NO: 65 - DNA, 81 bp, synthetic construct
  source 1..81: mol_type = other DNA; note = Description of Artificial Sequence: Synthetic oligonucleotide
ccaccggcaagctgcccgtgccctggcccaccctcgtgaccaccttcacctacggcgtgcagtgcttcgcccgctaccccg

SEQ ID NO: 66 - DNA, 81 bp, synthetic construct
  source 1..81: mol_type = other DNA; note = Description of Artificial Sequence: Synthetic oligonucleotide
cggggtagcgggcgaagcactgcacgccgtaggtgaaggtggtcacgagggtgggccagggcacgggcagcttgccggtgg

SEQ ID NO: 67 - DNA, 81 bp, synthetic construct
  source 1..81: mol_type = other DNA; note = Description of Artificial Sequence: Synthetic oligonucleotide
ccgtgccctggcccaccctcgtgaccaccttcacctacggcgtgcagtgcttcgcccgctaccccgaccacatgaagcagc

SEQ ID NO: 68 - DNA, 81 bp, synthetic construct
  source 1..81: mol_type = other DNA; note = Description of Artificial Sequence: Synthetic oligonucleotide
gctgcttcatgtggtcggggtagcgggcgaagcactgcacgccgtaggtgaaggtggtcacgagggtgggccagggcacgg

SEQ ID NO: 69 - DNA, 98 bp, synthetic construct
  source 1..98: mol_type = other DNA; note = Description of Artificial Sequence: Synthetic oligonucleotide
ccaccggcaagctgcccgtgccctggcccaccctcgtgaccaccttcacctacggcgtgcagtgcttcgcccgctaccccgaccacatgaagcagcac

SEQ ID NO: 70 - DNA, 97 bp, synthetic construct
  source 1..97: mol_type = other DNA; note = Description of Artificial Sequence: Synthetic oligonucleotide
gtgctgcttcatgtggtcggggtagcgggcgaagcactgcacgccgtaggtgaaggtggcacgagggtgggccagggcacgggcagcttgccggtgg

SEQ ID NO: 71 - DNA, 82 bp, synthetic construct
  source 1..82: mol_type = other DNA; note = Description of Artificial Sequence: Synthetic oligonucleotide
caagctgcccgtgccctggcccaccctcgtgaccaccttcacctacggcgtgcagtgcttcgcccgctaccccgaccacatg

SEQ ID NO: 72 - DNA, 82 bp, synthetic construct
  source 1..82: mol_type = other DNA; note = Description of Artificial Sequence: Synthetic oligonucleotide
catgtggtcggggtagcgggcgaagcactgcacgccgtaggtgaaggtggtcacgagggtgggccagggcacgggcagcttg

SEQ ID NO: 73 - skipped

SEQ ID NO: 74 - DNA, 99 bp, synthetic construct
  source 1..99: mol_type = other DNA; note = Description of Artificial Sequence: Synthetic oligonucleotide
gtgccctggcccaccctcgtgaccaccctgaccgactacaaagacgatgacgacaagaattcttacggcgtgcagtgcttcagccgctaccccgaccac

SEQ ID NO: 75 - DNA, 31 bp, synthetic construct
  source 1..31: mol_type = other DNA; note = Description of Artificial Sequence: Synthetic oligonucleotide
gactacaaagacgatgacgacaagaattctt

SEQ ID NO: 76 - DNA, 31 bp, synthetic construct
  source 1..31: mol_type = other DNA; note = Description of Artificial Sequence: Synthetic oligonucleotide
aagaattcttgtcgtcatcgtctttgtagtc

SEQ ID NO: 77 - DNA, 37 bp, synthetic construct
  source 1..37: mol_type = other DNA; note = Description of Artificial Sequence: Synthetic oligonucleotide
ctgaccgactacaaagacgatgacgacaagaattctt

SEQ ID NO: 78 - DNA, 37 bp, synthetic construct
  source 1..37: mol_type = other DNA; note = Description of Artificial Sequence: Synthetic oligonucleotide
cgccgtaagaattcttgtcgtcatcgtctttgtagtc

SEQ ID NO: 79 - DNA, 37 bp, synthetic construct
  source 1..37: mol_type = other DNA; note = Description of Artificial Sequence: Synthetic oligonucleotide
gactacaaagacgatgacgacaagaattcttacggcg

SEQ ID NO: 80 - DNA, 37 bp, synthetic construct
  source 1..37: mol_type = other DNA; note = Description of Artificial Sequence: Synthetic oligonucleotide
aagaattcttgtcgtcatcgtctttgtagtcggtcag

SEQ ID NO: 81 - DNA, 46 bp, synthetic construct
  source 1..46: mol_type = other DNA; note = Description of Artificial Sequence: Synthetic oligonucleotide
gtgaccaccctgaccgactacaaagacgatgacgacaagaattctt

SEQ ID NO: 82 - DNA, 45 bp, synthetic construct
  source 1..45: mol_type = other DNA; note = Description of Artificial Sequence: Synthetic oligonucleotide
gcactgcacgccgtaagaattcttgtcgtcatcgtctttgtagtc

SEQ ID NO: 83 - DNA, 45 bp, synthetic construct
  source 1..45: mol_type = other DNA; note = Description of Artificial Sequence: Synthetic oligonucleotide
gactacaaagacgatgacgacaagaattcttacggcgtgcagtgc

SEQ ID NO: 84 - DNA, 46 bp, synthetic construct
  source 1..46: mol_type = other DNA; note = Description of Artificial Sequence: Synthetic oligonucleotide
aagaattcttgtcgtcatcgtctttgtagtcggtcagggtggtcac

SEQ ID NO: 85 - DNA, 64 bp, synthetic construct
  source 1..64: mol_type = other DNA; note = Description of Artificial Sequence: Synthetic oligonucleotide
gtgccctggcccaccctcgtgaccaccctgaccgactacaaagacgatgacgacaagaattctt

SEQ ID NO: 86 - DNA, 66 bp, synthetic construct
  source 1..66: mol_type = other DNA; note = Description of Artificial Sequence: Synthetic oligonucleotide
gtggtcggggtagcggctgaagcactgcacgccgtaagaattcttgtcgtcatcgtctttgtagtc

SEQ ID NO: 87 - DNA, 66 bp, synthetic construct
  source 1..66: mol_type = other DNA; note = Description of Artificial Sequence: Synthetic oligonucleotide
gactacaaagacgatgacgacaagaattcttacggcgtgcagtgcttcagccgctaccccgaccac

SEQ ID NO: 88 - DNA, 64 bp, synthetic construct
  source 1..64: mol_type = other DNA; note = Description of Artificial Sequence: Synthetic oligonucleotide
aagaattcttgtcgtcatcgtctttgtagtcggtcagggtggtcacgagggtgggccagggcac

SEQ ID NO: 89 - DNA, 60 bp, synthetic construct
  source 1..60: mol_type = other DNA; note = Description of Artificial Sequence: Synthetic oligonucleotide
gactacaaagacgatgacgacaagaattcttacggcgtgcagtgcttcagccgctacccc

SEQ ID NO: 90 - DNA, 58 bp, synthetic construct
  source 1..58: mol_type = other DNA; note = Description of Artificial Sequence: Synthetic oligonucleotide
aagaattcttgtcgtcatcgtctttgtagtcggtcagggtggtcacgagggtgggcca

SEQ ID NO: 91 - DNA, 66 bp, synthetic construct; identical to SEQ ID NO: 87
  source 1..66: mol_type = other DNA; note = Description of Artificial Sequence: Synthetic oligonucleotide

SEQ ID NO: 92 - DNA, 64 bp, synthetic construct; identical to SEQ ID NO: 88
  source 1..64: mol_type = other DNA; note = Description of Artificial Sequence: Synthetic oligonucleotide

SEQ ID NO: 93 - DNA, 67 bp, synthetic construct
  source 1..67: mol_type = other DNA; note = Description of Artificial Sequence: Synthetic oligonucleotide
aagaattcttgtcgtcatcgtctttgtagtcggtcagggtggtcacgagggtgggccagggcacggg

SEQ ID NO: 94 - DNA, 66 bp, synthetic construct; identical to SEQ ID NO: 87
  source 1..66: mol_type = other DNA; note = Description of Artificial Sequence: Synthetic oligonucleotide

SEQ ID NO: 95 - DNA, 78 bp, synthetic construct
  source 1..78: mol_type = other DNA; note = Description of Artificial Sequence: Synthetic oligonucleotide
gactacaaagacgatgacgacaagaattcttacggcgtgcagtgcttcagccgctaccccgaccacatgaagcagcac

SEQ ID NO: 96 - DNA, 78 bp, synthetic construct
  source 1..78: mol_type = other DNA; note = Description of Artificial Sequence: Synthetic oligonucleotide
aagaattcttgtcgtcatcgtctttgtagtcggtcagggtggtcacgagggtgggccagggcacgggcagcttgccgg

SEQ ID NO: 97 - DNA, 94 bp, synthetic construct
  source 1..94: mol_type = other DNA; note = Description of Artificial Sequence: Synthetic oligonucleotide
gcccgtgccctggcccaccctcgtgaccacctgactacaaagacgatgacgacaagaattctacggcgtgcagtgcttcgcccgctaccccgac

SEQ ID NO: 98 - DNA, 63 bp, synthetic construct
  source 1..63: mol_type = other DNA; note = Description of Artificial Sequence: Synthetic oligonucleotide
gcccgtgccctggcccaccctcgtgaccacctgactacaaagacgatgacgacaagaattcta

SEQ ID NO: 99 - DNA, 62 bp, synthetic construct
  source 1..62: mol_type = other DNA; note = Description of Artificial Sequence: Synthetic oligonucleotide
gtcggggtagcgggcgaagcactgcacgccgtagaattcttgtcgtcatcgtctttgtagtc

SEQ ID NO: 100 - DNA, 62 bp, synthetic construct
  source 1..62: mol_type = other DNA; note = Description of Artificial Sequence: Synthetic oligonucleotide
agaattcttgtcgtcatcgtctttgtagtcaggtggtcacgagggtgggccagggcacgggc

SEQ ID NO: 101 - DNA, 62 bp, synthetic construct
  source 1..62: mol_type = other DNA; note = Description of Artificial Sequence: Synthetic oligonucleotide
gactacaaagacgatgacgacaagaattctacggcgtgcagtgcttcgcccgctaccccgac

SEQ ID NO: 102 - DNA, 23 bp, synthetic construct
  source 1..23: mol_type = other DNA; note = Description of Artificial Sequence: Synthetic primer
ctcgtgaccaccctgacccacgg

SEQ ID NO: 103 - DNA, 23 bp, synthetic construct
  source 1..23: mol_type = other DNA; note = Description of Artificial Sequence: Synthetic primer
ctgaagttcatctgcaccaccgg

SEQ ID NO: 104 - DNA, 23 bp, synthetic construct
  source 1..23: mol_type = other DNA; note = Description of Artificial Sequence: Synthetic primer
gggcacgggcagcttgccggtgg

SEQ ID NO: 105 - DNA, 23 bp, synthetic construct
  source 1..23: mol_type = other DNA; note = Description of Artificial Sequence: Synthetic primer
ccagggcacgggcagcttgccgg

SEQ ID NO: 106 - DNA, 21 bp, synthetic construct
  source 1..21: mol_type = other DNA; note = Description of Artificial Sequence: Synthetic primer
ggcaagctgcccgtgccctgg

SEQ ID NO: 107 - DNA, 23 bp, synthetic construct
  source 1..23: mol_type = other DNA; note = Description of Artificial Sequence: Synthetic primer
cacgagggtgggccagggcacgg

SEQ ID NO: 108 - DNA, 23 bp, synthetic construct
  source 1..23: mol_type = other DNA; note = Description of Artificial Sequence: Synthetic primer
ggtggtcacgagggtgggccagg

SEQ ID NO: 109 - DNA, 23 bp, synthetic construct
  source 1..23: mol_type = other DNA; note = Description of Artificial Sequence: Synthetic primer
gccgtaggtggtcacgagggtgg

SEQ ID NO: 110 - DNA, 23 bp, synthetic construct
  source 1..23: mol_type = other DNA; note = Description of Artificial Sequence: Synthetic primer
gcacgccgtaggtggtcacgagg

SEQ ID NO: 111 - DNA, 23 bp, synthetic construct
  source 1..23: mol_type = other DNA; note = Description of Artificial Sequence: Synthetic primer
cccaccctcgtgaccacctacgg

SEQ ID NO: 112 - DNA, 23 bp, synthetic construct
  source 1..23: mol_type = other DNA; note = Description of Artificial Sequence: Synthetic primer
gaagcactgcacgccgtaggtgg

SEQ ID NO: 113 - DNA, 23 bp, synthetic construct
  source 1..23: mol_type = other DNA; note = Description of Artificial Sequence: Synthetic primer
ggcgaagcactgcacgccgtagg

SEQ ID NO: 114 - DNA, 23 bp, synthetic construct
  source 1..23: mol_type = other DNA; note = Description of Artificial Sequence: Synthetic primer
cttcatgtggtcggggtagcggg

SEQ ID NO: 115 - DNA, 23 bp, synthetic construct
  source 1..23: mol_type = other DNA; note = Description of Artificial Sequence: Synthetic primer
gtcgtgctgcttcatgtggtcgg

SEQ ID NO: 116 - DNA, 23 bp, synthetic construct
  source 1..23: mol_type = other DNA; note = Description of Artificial Sequence: Synthetic primer
agaagtcgtgctgcttcatgtgg

SEQ ID NO: 117 - DNA, 23 bp, synthetic construct
  source 1..23: mol_type = other DNA; note = Description of Artificial Sequence: Synthetic primer
gcatttctcagtcctaaacaggg

SEQ ID NO: 118 - DNA, 20 bp, synthetic construct
  source 1..20: mol_type = other DNA; note = Description of Artificial Sequence: Synthetic primer
agcggctctagtatcaaccc

SEQ ID NO: 119 - DNA, 20 bp, synthetic construct
  source 1..20: mol_type = other DNA; note = Description of Artificial Sequence: Synthetic primer
aagatatgtagccgccctac

SEQ ID NO: 120 - DNA, 20 bp, synthetic construct
  source 1..20: mol_type = other DNA; note = Description of Artificial Sequence: Synthetic primer
ccggtcaatgagcactattt

SEQ ID NO: 121 - DNA, 720 bp, synthetic construct
  source 1..720: mol_type = other DNA; note = Description of Artificial Sequence: Synthetic polynucleotide
atggtgagcaagggcgaggagctgttcaccggggtggtgcccatcctggtcgagctggacggcgacgtaaacggccacaagttcagcgtgtccggcgagggcgagggcgatgccacctacggcaagctgaccctgaagttcatctgcaccaccggcaagctgcccgtgccctggcccaccctcgtgaccaccttcacctacggcgtgcagtgcttcgcccgctaccccgaccacatgaagcagcacgacttcttcaagtccgccatgcccgaaggctacgtccaggagcgcaccatcttcttcaaggacgacggcaactacaagacccgcgccgaggtgaagttcgagggcgacaccctggtgaaccgcatcgagctgaagggcatcgacttcaaggaggacggcaacatcctggggcacaagctggagtacaactacaacagccacaaggtctatatcaccgccgacaagcagaagaacggcatcaaggtgaacttcaagacccgccacaacatcgaggacggcagcgtgcagctcgccgaccactaccagcagaacacccccatcggcgacggccccgtgctgctgcccgacaaccactacctgagcacccagtccgccctgagcaaagaccccaacgagaagcgcgatcacatggtcctgctggagttcgtgaccgccgccgggatcactctcggcatggacgagctgtacaagtaa

SEQ ID NO: 122 - DNA, 714 bp, synthetic construct
  source 1..714: mol_type = other DNA; note = Description of Artificial Sequence: Synthetic polynucleotide
atggtgagcaagggcgaggagctgttcaccggggtggtgcccatcctggtcgagctggacggcgacgtaaacggccacaagttcagcgtgtccggcgagggcgagggcgatgccacctacggcaagctgaccctgaagttcatctgcaccaccggcaagctgcccgtgccctggcccaccctcgtgaccacctacggcgtgcagtgcttcgcccgctaccccgaccacatgaagcagcacgacttcttcaagtccgccatgcccgaaggctacgtccaggagcgcaccatcttcttcaaggacgacggcaactacaagacccgcgccgaggtgaagttcgagggcgacaccctggtgaaccgcatcgagctgaagggcatcgacttcaaggaggacggcaacatcctggggcacaagctggagtacaactacaacagccacaaggtctatatcaccgccgacaagcagaagaacggcatcaaggtgaacttcaagacccgccacaacatcgaggacggcagcgtgcagctcgccgaccactaccagcagaacacccccatcggcgacggccccgtgctgctgcccgacaaccactacctgagcacccagtccgccctgagcaaagaccccaacgagaagcgcgatcacatggtcctgctggagttcgtgaccgccgccgggatcactctcggcatggacgagctgtacaagtaa

SEQ ID NO: 123 - DNA, 720 bp, synthetic construct
  source 1..720: mol_type = other DNA; note = Description of Artificial Sequence: Synthetic polynucleotide
atggtgagcaagggcgaggagctgttcaccggggtggtgcccatcctggtcgagctggacggcgacgtaaacggccacaagttcagcgtgtccggcgagggcgagggcgatgccacctacggcaagctgaccctgaagttcatctgcaccaccggcaagctgcccgtgccctggcccaccctcgtgaccaccctgacccacggcgtgcagtgcttcagccgctaccccgaccacatgaagcagcacgacttcttcaagtccgccatgcccgaaggctacgtccaggagcgcaccatcttcttcaaggacgacggcaactacaagacccgcgccgaggtgaagttcgagggcgacaccctggtgaaccgcatcgagctgaagggcatcgacttcaaggaggacggcaacatcctggggcacaagctggagtacaactacaacagccacaacgtctatatcatggccgacaagcagaagaacggcatcaaggtgaacttcaagatccgccacaacatcgaggacggcagcgtgcagctcgccgaccactaccagcagaacacccccatcggcgacggccccgtgctgctgcccgacaaccactacctgagcacccagtccgccctgagcaaagaccccaacgagaagcgcgatcacatggtcctgctggagttcgtgaccgccgccgggatcactctcggcatggacgagctgtacaagtaa

SEQ ID NO: 124 - DNA, 720 bp, synthetic construct
  source 1..720: mol_type = other DNA; note = Description of Artificial Sequence: Synthetic polynucleotide
atggtgagcaagggcgaggagctgttcaccggggtggtgcccatcctggtcgagctggacggcgacgtaaacggccacaagttcagcgtgtccggcgagggcgagggcgatgccacctacggcaagctgaccctgaagttcatctgcaccaccggcaagctgcccgtgccctggcccaccctcgtgaccaccctgacctacggcgtgcagtgcttcagccgctaccccgaccacatgaagcagcacgacttcttcaagtccgccatgcccgaaggctacgtccaggagcgcaccatcttcttcaaggacgacggcaactacaagacccgcgccgaggtgaagttcgagggcgacaccctggtgaaccgcatcgagctgaagggcatcgacttcaaggaggacggcaacatcctggggcacaagctggagtacaactacaacagccacaacgtctatatcatggccgacaagcagaagaacggcatcaaggtgaacttcaagatccgccacaacatcgaggacggcagcgtgcagctcgccgaccactaccagcagaacacccccatcggcgacggccccgtgctgctgcccgacaaccactacctgagcacccagtccgccctgagcaaagaccccaacgagaagcgcgatcacatggtcctgctggagttcgtgaccgccgccgggatcactctcggcatggacgagctgtacaagtaa

SEQ ID NO: 125 - DNA, 23 bp, synthetic construct
  source 1..23: mol_type = other DNA; note = Description of Artificial Sequence: Synthetic oligonucleotide
ctcgtgaccaccttcacctacgg

SEQ ID NO: 126 - DNA, 24 bp, synthetic construct
  source 1..24: mol_type = other DNA; note = Description of Artificial Sequence: Synthetic primer
atggtgagcaagggcgaggagctg

SEQ ID NO: 127 - DNA, 22 bp, synthetic construct
  source 1..22: mol_type = other DNA; note = Description of Artificial Sequence: Synthetic primer
gtcctccttgaagtcgatgccc